European Patent Specification EP 3 045 531 B1, published August 30, 2023. Title: A method for inducing differentiation of induced pluripotent stem cell and a method for selection of induced pluripotent stem cell. Applicant: Kaneka Corporation. The sequence listing filed with the application follows.

SEQUENCE LISTING (16 sequences)

SEQ ID NO: 1 - DNA, 20 bp, Artificial Sequence
  Description of Artificial Sequence: primer
accacagtccatgccatcac

SEQ ID NO: 2 - DNA, 20 bp, Artificial Sequence
  Description of Artificial Sequence: primer
tccaccaccctgttgctgta

SEQ ID NO: 3 - DNA, 20 bp, Artificial Sequence
  Description of Artificial Sequence: primer
ttttgggacccgaactttcc

SEQ ID NO: 4 - DNA, 23 bp, Artificial Sequence
  Description of Artificial Sequence: primer
ctcctggtatcctttagcaactc

SEQ ID NO: 5 - DNA, 24 bp, Artificial Sequence
  Description of Artificial Sequence: primer
gcacaccagtccaacagcaccaat

SEQ ID NO: 6 - DNA, 25 bp, Artificial Sequence
  Description of Artificial Sequence: primer
ccgaagttgacagtgaaggcttctg

SEQ ID NO: 7 - DNA, 20 bp, Artificial Sequence
  Description of Artificial Sequence: primer
ggtgttgattgcctttgctc

SEQ ID NO: 8 - DNA, 20 bp, Artificial Sequence
  Description of Artificial Sequence: primer
cccttcatcccgaagttcat

SEQ ID NO: 9 - DNA, 20 bp, Artificial Sequence
  Description of Artificial Sequence: primer
ctcccaaggcacagagacac

SEQ ID NO: 10 - DNA, 20 bp, Artificial Sequence
  Description of Artificial Sequence: primer
ggagccgtagtgagcagttc

SEQ ID NO: 11 - DNA, 20 bp, Artificial Sequence
  Description of Artificial Sequence: primer
cgaaaaagccacacattcct

SEQ ID NO: 12 - DNA, 20 bp, Artificial Sequence
  Description of Artificial Sequence: primer
cacggtacttgtccacgatg

SEQ ID NO: 13 - DNA, 20 bp, Artificial Sequence
  Description of Artificial Sequence: primer
aagagatccgcacgcagtat

SEQ ID NO: 14 - DNA, 20 bp, Artificial Sequence
  Description of Artificial Sequence: primer
gtaggtggcgatctcgatgt

SEQ ID NO: 15 - DNA, 20 bp, Artificial Sequence
  Description of Artificial Sequence: primer
tgcgggctactgaaaagttc

SEQ ID NO: 16 - DNA, 20 bp, Artificial Sequence
  Description of Artificial Sequence: primer
ggggagggaagttgggctca